European Patent Application EP 4 239 064 A1, published September 6, 2023. Title: MUTANT CIS-PRENYLTRANSFERASE (CPT) FAMILY PROTEIN, METHOD FOR PRODUCING POLYISOPRENOID, VECTOR, TRANSGENIC PLANT, METHOD FOR PRODUCING PNEUMATIC TIRE, AND METHOD FOR PRODUCING RUBBER PRODUCT. Applicant: SUMITOMO RUBBER INDUSTRIES, LTD. Application EP. The sequence listing filed with the application follows.

SEQUENCE LISTING (42 sequences)

SEQ ID NO: 1 - protein, 290 aa, Hevea brasiliensis
MELYNGERPSVFRLLGKYMRKGLYSILTQGPIPTHIAFILDGNRRFAKKHKLPEGGGHKAGFLALLNVLTYCYELGVKYATIYAFSIDNFRRKPHEVQYVMDLMLEKIEGMIMEESIINAYDICVRFVGNLKLLSEPVKTAADKIMRATANNSKCVLLIAVCYTSTDEIVHAVEESSELNSNEVCNNQELEEANATGSGTVIQIENMESYSGIKLVDLEKNTYINPYPDVLIRTSGETRLSNYLLWQTTNCILYSPHALWPEIGLRHVVWAVINFQRHYSYLEKHKEYLK

SEQ ID NO: 2 - DNA, 873 bp, Hevea brasiliensis
  source 1..873: mol_type = genomic DNA
atggaattatacaacggtgagaggccaagtgtgttcagacttttagggaagtatatgagaaaagggttatatagcatcctaacccagggtcccatccctactcatattgccttcatattggatggaaacaggaggtttgctaagaagcataaactgccagaaggaggtggtcataaggctggatttttagctcttctgaacgtactaacttattgctatgagttaggagtgaaatatgcgactatctatgcctttagcatcgataattttcgaaggaaacctcatgaggttcagtacgtaatggatctaatgctggagaagattgaagggatgatcatggaagaaagtatcatcaatgcatatgatatttgcgtacgttttgtgggtaacctgaagcttttaagtgagccagtcaagaccgcagcagataagattatgagggctactgccaacaattccaaatgtgtgcttctcattgctgtatgctatacttcaactgatgagatcgtgcatgctgttgaagaatcctctgaattgaactccaatgaagtttgtaacaatcaagaattggaggaggcaaatgcaactggaagcggtactgtgattcaaattgagaacatggagtcgtattctggaataaaacttgtagaccttgagaaaaacacctacataaatccttatcctgatgttctgattcgaacttctggggagacccgtctgagcaactacttactttggcagactactaattgcatactgtattctcctcatgcactgtggccagagattggtcttcgacacgtggtgtgggcagtaattaacttccaacgtcattattcttacttggagaaacataaggaatacttaaaataa

SEQ ID NO: 3 - protein, 302 aa, Arabidopsis thaliana
MLSILSSLLSLLFLFIISCFFITSHFWFPLSLPKILGFIKITSSRDDYDNEQRDEGTYVVGVEELQRELMPRHVAVIMDGNRRWAKRAGLLTSQGHEAGAKRLIEFSELCFKLGIHTVSAFAFSTENWGRHKIEVKCLMSLIQHYLKSKIQYFQREETRVSVIGNLTKIPESLLRTVQEIEEATRSYKKKHLILAIDYSGRLDILRACKSIVKKSEKGLIREEDVDEALIERELLTNCTEFPSPDLLIRTSGEQRISNFFLWQLAYTELFFSPVLWPDFDKDKLLEALVSYQRRERRFGCRV

SEQ ID NO: 4 - protein, 368 aa, Hevea brasiliensis
MEIFEAGRPSVLASLGRFIRKCIFRILSIGPIPSHVAFIMDGNRRFAKKEKLEEGSGHRAGSLALMSTLKYCYELGVKYVTIYAFSIDNFRRRPDEVQLIMDLILEKIEGLLRDENVVNAYGIRVRFVGTLKLLSEPVRVAAEKVARASAKNTKFVLVICIAYSSTDEIVHAVQESCKYKLNKIEPSNSNRACNDANEQVEENGKKIDSTITHGVQESCKDETDKSRTINAKPMYNGVTKEAGGTDNANTVIVNSIGDKWDDAHELEATRTGNGVISVEEIDKMLSHSSIKLVDIEKKLHMAVAPDPDILVRTSGESRLSNFLLWQTSNCSLYSPKALWPEIGLRHLVWAVITFQRNHSYLEKKKKQL

SEQ ID NO: 5 - DNA, 909 bp, Arabidopsis thaliana
  source 1..909: mol_type = genomic DNA
atgttgtctattctctcttctcttttatctctcctttttctgtttatcatctcttgtttcttcatcacaagccatttttggttccctctttccttgccaaaaatactcggattcatcaaaatcacatcttcgagagacgattatgacaacgagcaacgtgacgagggaacttatgtggtaggagtggaggagctacaaagagagctgatgccaagacatgtggcagtgataatggacggaaaccggagatgggccaaacgggccggattgctgacgtcacaaggccacgaggccggagctaaacggcttatagagttctccgagctttgctttaaattggggattcatacagtttcagcttttgccttctccacagagaattggggaagacacaagattgaggttaagtgcttgatgtctttgatccaacattacctcaagtccaagatccaatatttccaaagagaggaaactcgagtttctgttatcgggaacctaacgaagatccctgagtctctcctccgaacagtccaagagatagaggaagctacgagaagctataagaagaagcatctcatattggcaatagattacagcgggagattagacatcttgcgagcttgcaagagtattgtgaagaaatcagaaaaagggttgatccgagaggaagatgtagacgaggcattgatcgaaagagagcttctgacaaattgtactgagttcccaagtcctgatctattgattaggacaagtggagaacagaggattagtaacttcttcttgtggcaacttgcttatacagagctcttcttctcgccggtcctttggcctgatttcgataaggataagcttctagaggccctggtttcgtatcagcgccgggaaagacgatttggctgtcgggtttga

SEQ ID NO: 6 - DNA, 1107 bp, Hevea brasiliensis
  source 1..1107: mol_type = genomic DNA
atggaaatatttgaggctggtaggccaagcgtgcttgcaagtttggggagatttatcagaaaatgcatatttcgcattctatcaataggtcccatcccaagtcatgttgccttcataatggatggaaaccggaggtttgctaagaaggagaaactggaagaaggatctggtcacagggctggatctttagctctaatgtccacgcttaagtactgctatgagttgggagtgaagtatgtgactatatatgccttcagcattgataattttagaaggcgacctgatgaggttcagctcataatggatctaatactggagaagattgaggggctgctcagggacgaaaatgttgtcaatgcatatggcatcagagtacgatttgtaggtaccttgaagcttctaagtgagccagtcagggtcgcagcagaaaaagtcgccagggctagtgccaagaataccaagtttgtgcttgtcatttgtatagcctattcttcaactgatgagattgtgcatgctgttcaagaatcttgtaaatataaattgaacaaaattgagccatctaactccaacagggcttgcaatgatgcgaatgaacaagtagaagaaaatggtaagaagatagatagtaccatcacacatggtgttcaagaatcctgcaaagatgaaacagataaatctcgcacaataaacgcaaagccaatgtataatggtgtgaccaaagaagctggagggactgacaatgctaatactgtgatagtaaattccatcggagacaagtgggatgatgctcacgaactggaggcaactagaactggcaatggtgtgatttcagtagaagaaattgataagatgctgtcacattctagcataaagctggtagacattgagaaaaaattgcacatggctgtagcccctgatcctgatatcttggttcgaacttctggagagagccgtctgagcaacttcctactttggcagactagtaactgttcactgtattctccaaaggcactgtggccggagattggcctacgccacttggtgtgggcagtaataaccttccaacgtaatcattcttatttggagaagaaaaagaagcagttgtaa

SEQ ID NO: 7 - protein, 306 aa, synthetic construct
MLSILSSLLSLLFLFIISCFFITSHFWFPLSLPKILGFIKITSSRDDYDNEQRDEGTYVVGVEELQRELMPRHVAVIMDGNRRWAKRAGLLTSQGHEAGAKRLIEFSELCFKLGIHTVSAFAFSTENWGRHKIEVKCLMSLIQHYLKSKIQYFQREETRVSVIGNLTKIPESLLRTVQEIEEATRSYKKKHLILAIDYSGRLDILRACKSIVKKSEKGLIREEDVDEALIERELLTNCTEFPSPDLLIRTSGEQRISNFFLWQLAYTELFFSPVLWPDIGLRHVVWAVINFQRHYSYLEKHKEYLK

SEQ ID NO: 8 - protein, 369 aa, synthetic construct
MEIFEAGRPSVLASLGRFIRKCIFRILSIGPIPSHVAFIMDGNRRFAKKEKLEEGSGHRAGSLALMSTLKYCYELGVKYVTIYAFSIDNFRRRPDEVQLIMDLILEKIEGLLRDENVVNAYGIRVRFVGTLKLLSEPVRVAAEKVARASAKNTKFVLVICIAYSSTDEIVHAVQESCKYKLNKIEPSNSNRACNDANEQVEENGKKIDSTITHGVQESCKDETDKSRTINAKPMYNGVTKEAGGTDNANTVIVNSIGDKWDDAHELEATRTGNGVISVEEIDKMLSHSSIKLVDIEKKLHMAVAPDPDILVRTSGESRLSNFLLWQTSNCSLYSPKALWPEIGLRHVVWAVINFQRHYSYLEKHKEYLK

SEQ ID NO: 9 - DNA, 921 bp, synthetic construct
  source 1..921: mol_type = other DNA
atgttgtctattctctcttctcttttatctctcctttttctgtttatcatctcttgtttcttcatcacaagccatttttggttccctctttccttgccaaaaatactcggattcatcaaaatcacatcttcgagagacgattatgacaacgagcaacgtgacgagggaacttatgtggtaggagtggaggagctacaaagagagctgatgccaagacatgtggcagtgataatggacggaaaccggagatgggccaaacgggccggattgctgacgtcacaaggccacgaggccggagctaaacggcttatagagttctccgagctttgctttaaattggggattcatacagtttcagcttttgccttctccacagagaattggggaagacacaagattgaggttaagtgcttgatgtctttgatccaacattacctcaagtccaagatccaatatttccaaagagaggaaactcgagtttctgttatcgggaacctaacgaagatccctgagtctctcctccgaacagtccaagagatagaggaagctacgagaagctataagaagaagcatctcatattggcaatagattacagcgggagattagacatcttgcgagcttgcaagagtattgtgaagaaatcagaaaaagggttgatccgagaggaagatgtagacgaggcattgatcgaaagagagcttctgacaaattgtactgagttcccaagtcctgatctattgattaggacaagtggagaacagaggattagtaacttcttcttgtggcaacttgcttatacagagctcttcttctcgccggtcctttggcctgatattggtcttcgacacgtggtgtgggcagtaattaacttccaacgtcattattcttacttggagaaacataaggaatacttaaaataa

SEQ ID NO: 10 - DNA, 1110 bp, synthetic construct
  source 1..1110: mol_type = other DNA
atggaaatatttgaggctggtaggccaagcgtgcttgcaagtttggggagatttatcagaaaatgcatatttcgcattctatcaataggtcccatcccaagtcatgttgccttcataatggatggaaaccggaggtttgctaagaaggagaaactggaagaaggatctggtcacagggctggatctttagctctaatgtccacgcttaagtactgctatgagttgggagtgaagtatgtgactatatatgccttcagcattgataattttagaaggcgacctgatgaggttcagctcataatggatctaatactggagaagattgaggggctgctcagggacgaaaatgttgtcaatgcatatggcatcagagtacgatttgtaggtaccttgaagcttctaagtgagccagtcagggtcgcagcagaaaaagtcgccagggctagtgccaagaataccaagtttgtgcttgtcatttgtatagcctattcttcaactgatgagattgtgcatgctgttcaagaatcttgtaaatataaattgaacaaaattgagccatctaactccaacagggcttgcaatgatgcgaatgaacaagtagaagaaaatggtaagaagatagatagtaccatcacacatggtgttcaagaatcctgcaaagatgaaacagataaatctcgcacaataaacgcaaagccaatgtataatggtgtgaccaaagaagctggagggactgacaatgctaatactgtgatagtaaattccatcggagacaagtgggatgatgctcacgaactggaggcaactagaactggcaatggtgtgatttcagtagaagaaattgataagatgctgtcacattctagcataaagctggtagacattgagaaaaaattgcacatggctgtagcccctgatcctgatatcttggttcgaacttctggagagagccgtctgagcaacttcctactttggcagactagtaactgttcactgtattctccaaaggcactgtggccggagattggtcttcgacacgtggtgtgggcagtaattaacttccaacgtcattattcttacttggagaaacataaggaatacttaaaataa

SEQ ID NO: 11 - DNA, 774 bp, Hevea brasiliensis
  source 1..774: mol_type = genomic DNA
atggatttgaaacctggagctggagggcagagagttaatcgtttagtggatccgattagttatcattttcttcaatttctgtggcgtactctacatcttcttgtcagcttatggtaccttcaagttagtatggtccaaatgatcgaaggctttctaatctctagtggacttgtgaaacgctatggagccctcgatattgacaaggtccggtaccttgccattgtggtagatagtgaagaagcttaccaaatttctaaagttattcagcttttgaaatgggtggaagatatgggtgtgaaacatttatgcctctatgattcaaaaggagttctcaagacaaacaagaaaaccatcatggagagtttgaacaatgctatgccatttgaggaagcagttgaaaaagatgttttactggaccagaaacagatgactgtggaatttgcttccagctccgatggaaaggaagcaataaccagggcagctaacgtactctttatgaagtatttgaagtatgctaaaactggtgtaggaaaggaagaaccatgctttacagaagatcaaatggatgaggcactaaaagctataggttacaaagggccggaacctgacttgctattaatttatggacctgttagatgccatctaggtttctcaccgtggagacttcgatatactgagatggtgcatatgggacccttgaggtacatgaacctcggttcactaaaaaaggccattcacaggttcacaacagtgcagcaaaattatggtacatga

SEQ ID NO: 12 - protein, 257 aa, Hevea brasiliensis
MDLKPGAGGQRVNRLVDPISYHFLQFLWRTLHLLVSLWYLQVSMVQMIEGFLISSGLVKRYGALDIDKVRYLAIVVDSEEAYQISKVIQLLKWVEDMGVKHLCLYDSKGVLKTNKKTIMESLNNAMPFEEAVEKDVLLDQKQMTVEFASSSDGKEAITRAANVLFMKYLKYAKTGVGKEEPCFTEDQMDEALKAIGYKGPEPDLLLIYGPVRCHLGFSPWRLRYTEMVHMGPLRYMNLGSLKKAIHRFTTVQQNYGT

SEQ ID NO: 13 - DNA, 417 bp, Hevea brasiliensis
  source 1..417: mol_type = genomic DNA
atggctgaagacgaagacaaccaacaagggcagggggaggggttaaaatatttgggttttgtgcaagacgcggcaacttatgctgtgactaccttctcaaacgtctatctttttgccaaagacaaatctggtccactgcagcctggtgtcgatatcattgagggtccggtgaagaacgtggctgtacctctctataataggttcagttatattcccaatggagctctcaagtttgtagacagcacggttgttgcatctgtcactattatagatcgctctcttcccccaattgtcaaggacgcatctatccaagttgtttcagcaattcgagctgccccagaagctgctcgttctctggcttcttctttgcctgggcagaccaagatacttgctaaggtgttttatggagagaattga

SEQ ID NO: 14 - protein, 138 aa, Hevea brasiliensis
MAEDEDNQQGQGEGLKYLGFVQDAATYAVTTFSNVYLFAKDKSGPLQPGVDIIEGPVKNVAVPLYNRFSYIPNGALKFVDSTVVASVTIIDRSLPPIVKDASIQVVSAIRAAPEAARSLASSLPGQTKILAKVFYGEN

SEQ ID NO: 15 - DNA, 34 bp, synthetic construct
  misc_feature 1..34: note = PRIMER-1
  source 1..34: mol_type = other DNA
tttggatccgatggaattatacaacggtgagagg

SEQ ID NO: 16 - DNA, 39 bp, synthetic construct
  misc_feature 1..39: note = PRIMER-2
  source 1..39: mol_type = other DNA
tttgcggccgcttattttaagtattccttatgtttctcc

SEQ ID NO: 17 - DNA, 31 bp, synthetic construct
  misc_feature 1..31: note = PRIMER-3
  source 1..31: mol_type = other DNA
tttctcgagatggatttgaaacctggagctg

SEQ ID NO: 18 - DNA, 33 bp, synthetic construct
  misc_feature 1..33: note = PRIMER-4
  source 1..33: mol_type = other DNA
tttctcgagtcatgtaccataattttgctgcac

SEQ ID NO: 19 - DNA, 27 bp, synthetic construct
  misc_feature 1..27: note = PRIMER-5
  source 1..27: mol_type = other DNA
tttctcgagatggctgaagacgaagac

SEQ ID NO: 20 - DNA, 28 bp, synthetic construct
  misc_feature 1..28: note = PRIMER-6
  source 1..28: mol_type = other DNA
tttggatcctcaattctctccataaaac

SEQ ID NO: 21 - DNA, 32 bp, synthetic construct
  misc_feature 1..32: note = PRIMER-7
  source 1..32: mol_type = other DNA
gtgctggaattcatggaaatatttgaggctgg

SEQ ID NO: 22 - DNA, 61 bp, synthetic construct
  misc_feature 1..61: note = PRIMER-8
  source 1..61: mol_type = other DNA
aagcttgtcgacttaatggtgatggtgatgatgaccggtacgcaactgcttctttttcttc

SEQ ID NO: 23 - DNA, 46 bp, synthetic construct
  misc_feature 1..46: note = PRIMER-9
  source 1..46: mol_type = other DNA
acatcaccaagatatcatgttgtctattctctcttctcttttatct

SEQ ID NO: 24 - DNA, 26 bp, synthetic construct
  misc_feature 1..26: note = PRIMER-10
  source 1..26: mol_type = other DNA
gtcgaagaccaatatcaggccaaagg

SEQ ID NO: 25 - DNA, 36 bp, synthetic construct
  misc_feature 1..36: note = PRIMER-11
  source 1..36: mol_type = other DNA
acatcaccaagatatcatggaaatatttgaggctgg

SEQ ID NO: 26 - DNA, 20 bp, synthetic construct
  misc_feature 1..20: note = PRIMER-12
  source 1..20: mol_type = other DNA
gaagaccaatctccggccac

SEQ ID NO: 27 - DNA, 26 bp, synthetic construct
  misc_feature 1..26: note = PRIMER-13
  source 1..26: mol_type = other DNA
cctttggcctgatattggtcttcgac

SEQ ID NO: 28 - DNA, 27 bp, synthetic construct
  misc_feature 1..27: note = PRIMER-14
  source 1..27: mol_type = other DNA
tacaggttttcctcgagttattttaag

SEQ ID NO: 29 - DNA, 20 bp, synthetic construct
  misc_feature 1..20: note = PRIMER-15
  source 1..20: mol_type = other DNA
gtggccggagattggtcttc

SEQ ID NO: 30 - DNA, 27 bp, synthetic construct
  misc_feature 1..27: note = PRIMER-16
  source 1..27: mol_type = other DNA
tacaggttttcctcgagttattttaag

SEQ ID NO: 31 - DNA, 46 bp, synthetic construct; identical to SEQ ID NO: 23
  misc_feature 1..46: note = PRIMER-17
  source 1..46: mol_type = other DNA

SEQ ID NO: 32 - DNA, 28 bp, synthetic construct
  misc_feature 1..28: note = PRIMER-18
  source 1..28: mol_type = other DNA
tgattggccgaggcggccttattttaag

SEQ ID NO: 33 - DNA, 36 bp, synthetic construct; identical to SEQ ID NO: 25
  misc_feature 1..36: note = PRIMER-19
  source 1..36: mol_type = other DNA

SEQ ID NO: 34 - DNA, 28 bp, synthetic construct
  misc_feature 1..28: note = PRIMER-20
  source 1..28: mol_type = other DNA
tgattggccgaggcggccttattttaag

SEQ ID NO: 35 - DNA, 46 bp, synthetic construct; identical to SEQ ID NO: 23
  misc_feature 1..46: note = PRIMER-21
  source 1..46: mol_type = other DNA

SEQ ID NO: 36 - DNA, 35 bp, synthetic construct
  misc_feature 1..35: note = PRIMER-22
  source 1..35: mol_type = other DNA
tgattggccgaggcggcctcaaacccgacagccaa

SEQ ID NO: 37 - DNA, 36 bp, synthetic construct; identical to SEQ ID NO: 25
  misc_feature 1..36: note = PRIMER-23
  source 1..36: mol_type = other DNA

SEQ ID NO: 38 - DNA, 39 bp, synthetic construct
  misc_feature 1..39: note = PRIMER-24
  source 1..39: mol_type = other DNA
tgattggccgaggcggcctacaactgcttctttttcttc

SEQ ID NO: 39 - DNA, 46 bp, synthetic construct; identical to SEQ ID NO: 23
  misc_feature 1..46: note = PRIMER-25
  source 1..46: mol_type = other DNA

SEQ ID NO: 40 - DNA, 28 bp, synthetic construct
  misc_feature 1..28: note = PRIMER-26
  source 1..28: mol_type = other DNA
tgattggccgaggcggccttattttaag

SEQ ID NO: 41 - DNA, 36 bp, synthetic construct; identical to SEQ ID NO: 25
  misc_feature 1..36: note = PRIMER-27
  source 1..36: mol_type = other DNA

SEQ ID NO: 42 - DNA, 28 bp, synthetic construct
  misc_feature 1..28: note = PRIMER-28
  source 1..28: mol_type = other DNA
tgattggccgaggcggccttattttaag